European Patent Specification EP 3 901 170 B1, published May 6, 2026. Title: RECOMBINANT ANTIBODY OF ANTI-HUMAN N-TERMINAL PRO-BRAIN NATRIURETIC PEPTIDE. Applicant: FAPON BIOTECH INC. The sequence listing filed with the application follows.

SEQUENCE LISTING (12 sequences)

SEQ ID NO: 1 - protein, 23 aa, Mus musculus
QAVLTQPSSVSRSLGQTVSITCS

SEQ ID NO: 2 - protein, 13 aa, Mus musculus
WFQLIPGSAPKTL

SEQ ID NO: 3 - protein, 31 aa, Mus musculus
VPDRFSGSRSGNTATLTINSLQAEDEADYYC

SEQ ID NO: 4 - protein, 13 aa, Mus musculus
SGTRLTVLSQPKS

SEQ ID NO: 5 - protein, 25 aa, Mus musculus
QVRLQESGPSQVKPAQTLSLTCAIS

SEQ ID NO: 6 - protein, 15 aa, Mus musculus
WVRHTPGKPPEWLAQ

SEQ ID NO: 7 - protein, 30 aa, Mus musculus
RLSITRDTSKSQVFLKLTGVTTEDTAVYYC

SEQ ID NO: 8 - protein, 9 aa, Mus musculus
PGLLVTVSS

SEQ ID NO: 9 - protein, 101 aa, Mus musculus
APSVTLFPPSKEELDTNKATVVCLISDFYPGSVNVVWKADGSTINQNVKTTQASKQSNSKYAASSYLTLTGSEWKSKSSYTCEVTHEGSTVTKTVKPSECS

SEQ ID NO: 10 - protein, 331 aa, Mus musculus
ASTTPPKVYPLTSCCGDTSSSIVTLGCLVSSYMPEPVTVTWNSGALTSGVHTFPAILQSSGLYSLSSVVTVPASTSGAQTFICNVAHPASSTKVDKRVEPGCPDPCKHCRCPPPELPGGPSVFIFPPKPKDTLTISGTPEVTCVVVDVGQDDPEVQFSWFVDNVEVRTARTKPREEQFNSTFRVVSALPIQHQDWTGGKEFKCKVHNEGLPAPIVRTISRTKGQAREPQVYVLAPPQEELSKSTLSVTCLVTGFYPDYIAVEWQKNGQPESEDKYGTTTSQLDADGSYFLYSRLRVDKNSWQEGDTYACVVMHEALHNHYTQKSISKPPGK

SEQ ID NO: 11 - protein, 216 aa, Artificial Sequence
  light chain
QAVLTQPSSVSRSLGQTVSITCSGSSDQVGFGDYINWFQLIPGSAPKTLIFGAYSRIRGVPDRFSGSRSGNTATLTINSLQAEDEADYYCGSPNSRGGYVFGSGTRLTVLSQPKSAPSVTLFPPSKEELDTNKATVVCLISDFYPGSVNVVWKADGSTINQNVKTTQASKQSNSKYAASSYLTLTGSEWKSKSSYTCEVTHEGSTVTKTVKPSECS

SEQ ID NO: 12 - protein, 443 aa, Artificial Sequence
  heavy chain
QVRLQESGPSQVKPAQTLSLTCAISGFSITTYYLDWVRHTPGKPPEWLAQMTKDGNAVHQPTVRSRLSITRDTSKSQVFLKLTGVTTEDTAVYYCVRGVIDFGPGLLVTVSSASTTPPKVYPLTSCCGDTSSSIVTLGCLVSSYMPEPVTVTWNSGALTSGVHTFPAILQSSGLYSLSSVVTVPASTSGAQTFICNVAHPASSTKVDKRVEPGCPDPCKHCRCPPPELPGGPSVFIFPPKPKDTLTISGTPEVTCVVVDVGQDDPEVQFSWFVDNVEVRTARTKPREEQFNSTFRVVSALPIQHQDWTGGKEFKCKVHNEGLPAPIVRTISRTKGQAREPQVYVLAPPQEELSKSTLSVTCLVTGFYPDYIAVEWQKNGQPESEDKYGTTTSQLDADGSYFLYSRLRVDKNSWQEGDTYACVVMHEALHNHYTQKSISKPPGK